European Patent Application EP 4 660 310 A1, published December 10, 2025. Title: 定点整合位点筛选方法、载体微粒、定点整合方法和微粒. Applicant: 深圳太力生物技术有限责任公司. Application CN. The sequence listing filed with the application follows.

SEQUENCE LISTING (33 sequences)

SEQ ID NO: 1 - DNA, 444 bp, synthetic construct
  source 1..444: mol_type = other DNA
taattctggcaactatcaaaggttcaccaaggaaggaattctttatttggtatctgcaagcgcctgggtgttccaatttctatctgcaaatgtttgttcctgcagacatgtctaactatggtggaaacagagaccagcctcagatgtcacactgtgacctgacctataaaagctgaactttacaaagcataagcttgggttcatgcctgagtgaaaccagactgagtttctcttgtctctccgactgcttgcttggtcctgtgctggctaaaatttccatgacagtaggggtgtaaattattcagttttagtttcccagaaaactaaaagtaagactgtcatatgacctaatgatttgacttctggggtcctttcaattagctgttgaaaggacaatagattactcatggccatttaaacaattcacagtagcaaaaaggtgag

SEQ ID NO: 2 - DNA, 660 bp, synthetic construct
  source 1..660: mol_type = other DNA
gatatcgtgatgacacagtccccactttctctgcctgtcacccctggcgaacctgcttctatctcttgccggtcctcccagagcctcctgtattccatcggctacaactacctggattggtacctgcagaagagcggccaatcccctcagctgctgatctacctgggctccaaccgggccagcggagtgcccgatagattctccggctccggatctggcaccgacttcacactgaagatcagcagagtggaagctgaggacgtgggcttttactactgcatgcaggctctgcagaccccctacaccttcggccagggaaccaagctggaaatcaagcggaccgtggccgctccttctgtgttcatctttcctccttccgacgagcagctgaaatctggcaccgcctccgttgtgtgcctgctgaacaacttctaccctagagaggccaaggtgcagtggaaggtcgacaacgccctgcagtctggcaactctcaagagtccgtgacagaacaggactctaaggactccacctactccctgtcctctaccctgaccctgtccaaggccgactacgagaagcacaaagtgtacgcctgcgaggtgacccaccagggcctgtcttcacccgtgaccaagagcttcaatagaggcgagtgttga

SEQ ID NO: 3 - DNA, 1359 bp, synthetic construct
  source 1..1359: mol_type = other DNA
gaggtgcagctggttgaatccggtggcggactggagcagccaggtggctccctgcggttgtcctgtgctggctctggcttcaccttccgggattacgctatgacctgggtccggcaggccccaggcaaaggcctggaatgggtctcttctatctctggcagcggcggcaacacctactacgccgactcagtgaagggcagattcaccatctcccgggacaactcgaaaaataccctgtacctgcagatgaactctctgagagccgaggatacagccgtgtactactgcgccaaggacagactgtccatcaccatcagacctagatactacggcctggatgtgtggggccagggcaccaccgtgacagtgtcgtctgcctctaccaagggcccctccgtgttccctctggccccttgctctagatccacctccgagtctaccgctgctttgggctgcctggtgaaagactacttccccgagcccgtgaccgtgtcttggaactccggcgctctgacgtctggcgtgcacacctttccagctgtgctgcagtcctccggcctgtactccctgtcttccgtggtgaccgtgccttcttcttccctcggaaccaaaacctatacatgcaacgtggaccacaagccttccaacaccaaggtggataagcgggtcgagtccaagtacggacctccttgtcctccttgccctgctcctgagttcctgggaggccctagcgtgtttctgtttccacccaagcctaaggacaccctgatgatctccaggacccctgaagtgacctgcgtggtggtggacgtgtctcaagaggaccctgaggtgcagttcaactggtacgtggatggcgtggaagtgcataacgctaagaccaagccccgcgaggaacagttcaactccacctacagagtggtgtccgtgctgacagtgctgcaccaggactggctgaacggcaaagagtacaagtgcaaggtcagcaacaagggcctgcctagctccatcgagaagaccatctccaaggccaagggccagcctcgggaacctcaggtgtacaccctgcctcccagccaagaagagatgaccaagaaccaggtaagcctcacctgtctggtcaagggattctacccctctgacatcgccgtggaatgggagtccaatggccaacccgaaaacaactataagacaacacctcctgtgctggactccgacggctccttcttcctgtactctcggctgactgtggacaagtctagatggcaggagggcaatgtgttctcctgttccgtgatgcacgaggccctgcacaaccactacacccagaagtctctgagcctgtccctgggcaagtga

SEQ ID NO: 4 - DNA, 657 bp, synthetic construct
  source 1..657: mol_type = other DNA
gagatcgtgctgacccagtctcctgctaccctgtctctgagccccggcgaaagggctacactgtcctgtagagcctccaagggcgtgtccacttctggctactcctatctgcactggtaccagcagaagcctggccaggcccctcggctgctgatctacctggcctcttacctggaatccggcgtgccagccagattctccggtagcggctctggcaccgacttcaccctgacaatctcctccctggaacccgaggattttgccgtgtactactgccagcattctcgggacctgcctctgaccttcggcggaggcaccaaagtggaaatcaagcggaccgtggccgctccttccgtgttcatcttccctccttctgacgaacaactgaagagcggaaccgcttctgtagtgtgcctgctgaacaacttctaccctagagaggccaaagtgcagtggaaggtggacaacgccctgcagtccggcaactcccaagagtctgtcaccgagcaggattctaaggactccacctacagcctgtcctctaccctgaccctcagcaaggccgactacgagaagcacaaggtgtacgcctgcgaggtgacccaccagggcctgagttctcccgtcaccaagtcctttaatagaggcgagtgttga

SEQ ID NO: 5 - DNA, 1344 bp, synthetic construct
  source 1..1344: mol_type = other DNA
caagtgcagctggtgcagtctggcgtggaagtgaagaaacccggagcttcagtcaaggtgtcttgcaaggcctccggctacaccttcaccaactactacatgtactgggtgcggcaggcccctggccaaggcctggagtggatgggcggcatcaacccttctaatggcggaaccaacttcaatgagaagttcaagaacagagtgaccctgaccaccgactcttccaccacaaccgcttacatggaactgaagtccctgcagttcgacgataccgccgtgtactactgcgccagaagggactaccgcttcgacatgggattcgattattggggccagggcaccaccgtgacagtgtcttctgcctctacaaaaggacccagcgtgtttcctctggctccttgcagccggtctacctccgagtctaccgctgctctgggctgcctggtcaaagactacttccctgaacctgtgaccgtgtcctggaacagcggcgctctcacatccggcgtccacacctttccagctgtgctgcagtcttctggcctgtactccctgtcctccgtggtgaccgtgcctagcagctctctgggcaccaagacctatacctgcaacgtggaccacaagccttccaacaccaaagtggacaagcgggtggaatccaagtacggaccaccttgtcctccctgccctgcccccgagttcctgggcggcccctctgtgttcctcttccctcccaagcctaaggataccctgatgatctctcggaccccagaggtgacatgtgtggtcgtggacgtgagccaagaggaccctgaggtgcagtttaactggtacgtggatggcgtggaagtgcacaacgccaaaaccaagccccgggaggaacagttcaactccacctacagagtggtgtctgtgctgaccgtactgcaccaggactggctgaacggcaaggagtacaagtgcaaggtgtccaacaagggcctgccttcttccatcgagaagaccatctccaaggccaaaggtcagcctagagagcctcaggtgtacaccctgcctccatcccaggaagagatgaccaagaaccaggtcagcctcacatgtctggtgaagggcttctacccctccgacatcgccgtggaatgggagagcaatggccagcctgagaacaactacaagacaactcctcctgtgctggactccgacggctccttcttcctgtactccagactgaccgtagataagtccagatggcaggagggcaacgtgttctcctgttctgtgatgcacgaggccctgcataaccactacacccagaagagcctgagtctgtctctgggcaagtga

SEQ ID NO: 6 - DNA, 4128 bp, synthetic construct
  source 1..4128: mol_type = other DNA
caagtaaaacctctacaaatgtggtatggctgattagccggctatcgtactcgagtcaacactcgcctctattgaagctcttggtcacgggtgaagacaggccctggtgggtcacctcgcaggcgtacactttgtgcttctcgtagtcggccttggacagggtcagggtagaggacagggagtaggtggagtccttagagtcctgttctgtcacggactcttgagagttgccagactgcagggcgttgtcgaccttccactgcaccttggcctctctagggtagaagttgttcagcaggcacacaacggaggcggtgccagatttcagctgctcgtcggaaggaggaaagatgaacacagaaggagcggccacggtccgcttgatttccagcttggttccctggccgaaggtgtagggggtctgcagagcctgcatgcagtagtaaaagcccacgtcctcagcttccactctgctgatcttcagtgtgaagtcggtgccagatccggagccggagaatctatcgggcactccgctggcccggttggagcccaggtagatcagcagctgaggggattggccgctcttctgcaggtaccaatccaggtagttgtagccgatggaatacaggaggctctgggaggaccggcaagagatagaagcaggttcgccaggggtgacaggcagagaaagtggggactgtgtcatcacgatatcacatctagcgcctctcagccacagcaggagcaggcccagcagctgagcaggcactctcatgtccatggtggcggcaagcttcgtgtcaaggacggtgactgcagaaaagacccatggaaaggaacagtctgttagtctgtcagctattatgtctggtggcgcgcgcggcagcaacgagtactgctcagactacactgccctccaccgttaacagcaccgcaacgggagttacctctgactcttatcagaacacaacaactcagctgcctgcatcttcttctgccgctgccttaagtcttccaaatgcgtcagcggtgcaagcccgctccccgagctcattttcagacacataccctaccgccacggccttgtgcggcacactggtggtggtgggcatcgtgctgtgcctaagtctggcctccactgttaggagcaaggagctgccgagcgaccatgagtcgctggaggcatgggagcagggctcggatgtagaagctccgccgctaccggagaagagcccatgtccggaacacgtacccgagattcgcgtggagatcccacgttatgtttaataaaaactgcgggcactggggacggtggtgttgtatatgtgaatttgtaaataataaatgagaccccatcctgtaaaaatacagagtccgtgtcagtctctgaaggacagtgtattggcatatagccaataaagagagttgtggcaaagagccatgttatggattagtaatggaaagtatcgtcaccaataggggagtggtcaataatggtcaataacccacacctataggctaagctataccatcacctataacatgaggaagcgggggtgtatagaccccaagccaaaaacagtatagcatgcataagaagccaagggggtgggcctatagactctataggcggtacttacgtcactcttggcacggggaatccgcgttccaatgcaccgttcccggccgcggaggctggatcggtcccggtgtcttctatggaggtcaaaacagcgtggatggcgtctccaggcgatctgacggttcactaaacgagctctgcttatatagacctcccaccgtacacgcctaccgcccatttgcgtcaatggggcggagttgttacgacattttggaaagtcccgttgattttggtgccaaaacaaactcccattgacgtcaatggggtggagacttggaaatccccgtgagtcaaaccgctatccacgcccattgatgtactgccaaaaccgcatcaccatggtaatagcgatgactaatacgtagatgtactgccaagtaggaaagtcccataaggtcatgtactgggcataatgccaggcgggccatttaccgtcattgacgtcaatagggggcgtacttggcatatgatacacttgatgtactgccaagtgggcagtttaccgtaaatactccacccattgacgtcaatggaaagtccctattggcgttactatgggaacatacgtcattattgacgtcaatgggcgggggtcgttgggcggtcagccaggcgggccatttaccgtaagttatgtaacgcggaactccatatatgggctatgaactaatgaccccgtaattgattactattaataactagtcaataatcaatgtcaacatggcggtaatgttggacatgagccaatataaatgtacatattatgatatggcggccgcatgatcctgacgacggagaccgcggtggttgaccagacaaacctacatcgcgaagcagcgcaaaacgcctaaccctaagcagattcttcatgcaattgtcggtcaagccttgccttgttgtagcttaaattttgctcgcgcactactcagcgacctccaacacacaagcagggagcagatactggcttaactatgcggcatcagagcagattgtactgagagtcgaccataggggatcgggagatctcccgatccgtcgacgtcaggtggcacttttcggggaaatgtgcgcggaacccctatttgtttatttttctaaatacattcaaatatgtatccgctcatgagacaataaccctgataaatgcttcaataatattgaaaaaggaagagtatgagtattcaacatttccgtgtcgcccttattcccttttttgcggcattttgccttcctgtttttgctcacccagaaacgctggtgaaagtaaaagatgctgaagatcagttgggtgcacgagtgggttacatcgaactggatctcaacagcggtaagatccttgagagttttcgccccgaagaacgttttccaatgatgagcacttttaaagttctgctatgtggcgcggtattatcccgtattgacgccgggcaagagcaactcggtcgccgcatacactattctcagaatgacttggttgagtactcaccagtcacagaaaagcatcttacggatggcatgacagtaagagaattatgcagtgctgccataaccatgagtgataacactgcggccaacttacttctgacaacgatcggaggaccgaaggagctaaccgcttttttgcacaacatgggggatcatgtaactcgccttgatcgttgggaaccggagctgaatgaagccataccaaacgacgagcgtgacaccacgatgcctgtagcaatggcaacaacgttgcgcaaactattaactggcgaactacttactctagcttcccggcaacaattaatagactggatggaggcggataaagttgcaggaccacttctgcgctcggcccttccggctggctggtttattgctgataaatctggagccggtgagcgtgggtctcgcggtatcattgcagcactggggccagatggtaagccctcccgtatcgtagttatctacaagagaaactcagtctggtttcactcaggcatgaacccaagcttatgctttgtaaagttcagcttttataggtcaggtcacagtgtgacatctgaggctggtctctgtttccaccatagttagacatgtctgcaggaacaaacatttgcagatagaaattggaacacccaggcgcttgcagataccaaataaagaattccttccttggtgaacctttgatagttgccagaattattccttaaggtagtttatgtgaatgtttgccttcccaagacaagaggaggggggcagagtgaactcagcacatgagtaaaacagtaactcactctgttttctaagcaatcctacagtttccaggcaggaaattctattagacaatcaaaacacagagtaatagtttgattttattaggtatgtaatatgtaagggcatatatatttcatcaccactgccaatggcagttctactatgtgtatgatcttatttcttaattatttaatttttctgtgtcttcaacacaactctactagacg

SEQ ID NO: 7 - DNA, 22 bp, synthetic construct
  source 1..22: mol_type = other DNA
agaccagcctcagatgtcacac

SEQ ID NO: 8 - DNA, 20 bp, synthetic construct
  source 1..20: mol_type = other DNA
aggcacacaacggaggcggt

SEQ ID NO: 9 - DNA, 43 bp, synthetic construct
  source 1..43: mol_type = other DNA
atgatcctgacgacggagaccgcggtggttgaccagacaaacc

SEQ ID NO: 10 - DNA, 3671 bp, synthetic construct
  source 1..3671: mol_type = other DNA
tgggtcacctcgcaggcgtacaccttgtgcttctcgtagtcggccttgctgagggtcagggtagaggacaggctgtaggtggagtccttagaatcctgctcggtgacagactcttgggagttgccggactgcagggcgttgtccaccttccactgcactttggcctctctagggtagaagttgttcagcaggcacactacagaagcggttccgctcttcagttgttcgtcagaaggagggaagatgaacacggaaggagcggccacggtccgcttgatttccactttggtgcctccgccgaaggtcagaggcaggtcccgagaatgctggcagtagtacacggcaaaatcctcgggttccagggaggagattgtcagggtgaagtcggtgccagagccgctaccggagaatctggctggcacgccggattccaggtaagaggccaggtagatcagcagccgaggggcctggccaggcttctgctggtaccagtgcagataggagtagccagaagtggacacgcccttggaggctctacaggacagtgtagccctttcgccggggctcagagacagggtagcaggagactgggtcagcacgatctcggctctgccagcccacagtagtggtagtagtagtagtagtgctcgcatggtggcggcaagcttcgtgtcaaggacggtgactgcagaaaagacccatggaaaggaacagtctgttagtctgtcagctattatgtctggtggcgcgcgcggcagcaacgagtactgctcagactacactgccctccaccgttaacagcaccgcaacgggagttacctctgactcttatcagaacacaacaactcagctgcctgcatcttcttctgccgctgccttaagtcttccaaatgcgtcagcggtgcaagcccgctccccgagctcattttcagacacataccctaccgccacggccttgtgcggcacactggtggtggtgggcatcgtgctgtgcctaagtctggcctccactgttaggagcaaggagctgccgagcgaccatgagtcgctggaggcatgggagcagggctcggatgtagaagctccgccgctaccggagaagagcccatgtccggaacacgtacccgagattcgcgtggagatcccacgttatgtttaataaaaactgcgggcactggggacggtggtgttgtatatgtgaatttgtaaataataaatgagaccccatcctgtaaaaatacagagtccgtgtcagtctctgaaggacagtgtattggcatatagccaataaagagagttgtggcaaagagccatgttatggattagtaatggaaagtatcgtcaccaataggggagtggtcaataatggtcaataacccacacctataggctaagctataccatcacctataacatgaggaagcgggggtgtatagaccccaagccaaaaacagtatagcatgcataagaagccaagggggtgggcctatagactctataggcggtacttacgtcactcttggcacggggaatccgcgttccaatgcaccgttcccggccgcggaggctggatcggtcccggtgtcttctatggaggtcaaaacagcgtggatggcgtctccaggcgatctgacggttcactaaacgagctctgcttatatagacctcccaccgtacacgcctaccgcccatttgcgtcaatggggcggagttgttacgacattttggaaagtcccgttgattttggtgccaaaacaaactcccattgacgtcaatggggtggagacttggaaatccccgtgagtcaaaccgctatccacgcccattgatgtactgccaaaaccgcatcaccatggtaatagcgatgactaatacgtagatgtactgccaagtaggaaagtcccataaggtcatgtactgggcataatgccaggcgggccatttaccgtcattgacgtcaatagggggcgtacttggcatatgatacacttgatgtactgccaagtgggcagtttaccgtaaatactccacccattgacgtcaatggaaagtccctattggcgttactatgggaacatacgtcattattgacgtcaatgggcgggggtcgttgggcggtcagccaggcgggccatttaccgtaagttatgtaacgcggaactccatatatgggctatgaactaatgaccccgtaattgattactattaataactagtcaataatcaatgtcaacatggcggtaatgttggacatgagccaatataaatgtacatattatgatatggcggccgcatgatcctgacgacggagaccgcggtggttgaccagacaaacctacatcgcgaagcagcgcaaaacgcctaaccctaagcagattcttcatgcaattgtcggtcaagccttgccttgttgtagcttaaattttgctcgcgcactactcagcgacctccaacacacaagcagggagcagatactggcttaactatgcggcatcagagcagattgtactgagagtcgaccataggggatcgggagatctcccgatccgtcgacgtcaggtggcacttttcggggaaatgtgcgcggaacccctatttgtttatttttctaaatacattcaaatatgtatccgctcatgagacaataaccctgataaatgcttcaataatattgaaaaaggaagagtatgagtattcaacatttccgtgtcgcccttattcccttttttgcggcattttgccttcctgtttttgctcacccagaaacgctggtgaaagtaaaagatgctgaagatcagttgggtgcacgagtgggttacatcgaactggatctcaacagcggtaagatccttgagagttttcgccccgaagaacgttttccaatgatgagcacttttaaagttctgctatgtggcgcggtattatcccgtattgacgccgggcaagagcaactcggtcgccgcatacactattctcagaatgacttggttgagtactcaccagtcacagaaaagcatcttacggatggcatgacagtaagagaattatgcagtgctgccataaccatgagtgataacactgcggccaacttacttctgacaacgatcggaggaccgaaggagctaaccgcttttttgcacaacatgggggatcatgtaactcgccttgatcgttgggaaccggagctgaatgaagccataccaaacgacgagcgtgacaccacgatgcctgtagcaatggcaacaacgttgcgcaaactattaactggcgaactacttactctagcttcccggcaacaattaatagactggatggaggcggataaagttgcaggaccacttctgcgctcggcccttccggctggctggtttattgctgataaatctggagccggtgagcgtgggtctcgcggtatcattgcagcactggggccagatggtaagccctcccgtatcgtagttatctacaagagaaactcagtctggtttcactcaggcatgaacccaagcttatgctttgtaaagttcagcttttataggtcaggtcacagtgtgacatctgaggctggtctctgtttccaccatagttagacatgtctgcaggaacaaacatttgcagatagaaattggaacacccaggcgcttgcagataccaaataaagaattccttcc

SEQ ID NO: 11 - DNA, 21 bp, synthetic construct
  source 1..21: mol_type = other DNA
ccttagaatcctgctcggtga

SEQ ID NO: 12 - DNA, 66 bp, synthetic construct
  source 1..66: mol_type = other DNA
ttttaccacaactgatagtgtaagaaaacaaactgaagtagatagtcacccacaccagagacaaag

SEQ ID NO: 13 - DNA, 828 bp, synthetic construct
  source 1..828: mol_type = other DNA
cacggcgagggcaccttcaccagcgatgtctcctcttacctggaagagcaggccgctaaagagttcatcgcctggctggtgaagggaggaggcggcggcggaggctctggcggaggcggctccggcggcggtggctccgctgagtccaaatacggccctccatgtcctccttgccctgctcctgaggctgctggcggaccctccgtgttcctgttccctcccaagcccaaggacaccctgatgatcagccggacccctgaagtgacctgtgtggtcgtggacgtgtctcaagaggaccctgaggtgcagtttaactggtacgtggatggcgtggaagtacataacgccaagaccaagcctcgggaggaacagttcaactccacctacagagtggtgtctgtgctgacagtgctccaccaggactggctgaacggcaaagagtacaagtgcaaggtctccaacaagggcctgccttcctccatcgagaagaccatctctaaggccaagggccagcctagagagcctcaagtgtacaccctgcctccctctcaggaagagatgaccaagaatcaggtgagcctgacctgcctggtcaagggcttctacccttctgatatcgccgtggaatgggagtctaatggccagcccgagaacaactacaaaaccacaccacctgtgctggactccgacggctccttcttcctgtactccagactgaccgtggacaagtctagatggcaggagggcaacgtgttctcctgctccgtgatgcacgaggccctgcacaaccactatacacagaagtccttgagcctgtctctgggctga

SEQ ID NO: 14 - DNA, 2876 bp, synthetic construct
  source 1..2876: mol_type = other DNA
tgcagccacactaagatggcaaatgccactcaactatacatttcaaatagttaaggtggtgaattaagcagtaaatattttaccacaactgatagtgtaagaaaacaaaccgtcgtgtagataactacgatacgggagggcttaccatctggccccagtgctgcaatgataccgcgagacccacgctcaccggctccagatttatcagcaataaaccagccagccggaagggccgagcgcagaagtggtcctgcaactttatccgcctccatccagtctattaattgttgccgggaagctagagtaagtagttcgccagttaatagtttgcgcaacgttgttgccattgctacaggcatcgtggtgtcacgctcgtcgtttggtatggcttcattcagctccggttcccaacgatcaaggcgagttacatgatcccccatgttgtgcaaaaaagcggttagctccttcggtcctccgatcgttgtcagaagtaagttggccgcagtgttatcactcatggttatggcagcactgcataattctcttactgtcatgccatccgtaagatgcttttctgtgactggtgagtactcaaccaagtcattctgagaatagtgtatgcggcgaccgagttgctcttgcccggcgtcaatacgggataataccgcgccacatagcagaactttaaaagtgctcatcattggaaaacgttcttcggggcgaaaactctcaaggatcttaccgctgttgagatccagttcgatgtaacccactcgtgcacccaactgatcttcagcatcttttactttcaccagcgtttctgggtgagcaaaaacaggaaggcaaaatgccgcaaaaaagggaataagggcgacacggaaatgttgaatactcatactcttcctttttcaatattattgaagcatttatcagggttattgtctcatgagcggatacatatttgaatgtatttagaaaaataaacaaataggggttccgcgcacatttccccgaaaagtgccacctgacgtcgacggatcgggagatctcccgatcccctatggtcgactctcagtacaatctgctctgatgccgcatagttaagccagtatctgctccctgcttgtgtgttggaggtcgctgagtagtgcgcgagcaaaatttaagctacaacaaggcaaggcttgaccgacaattgcatgaagaatctgcttagggttaggcgttttgcgctgcttcgcgatgtaggtttgtctggtcaaccaccgcggtctccgtcgtcaggatcatgacattgattattgactagttattaatagtaatcaattacggggtcattagttcatagcccatatatggagttccgcgttacataacttacggtaaatggcccgcctggctgaccgcccaacgacccccgcccattgacgtcaataatgacgtatgttcccatagtaacgccaatagggactttccattgacgtcaatgggtggagtatttacggtaaactgcccacttggcagtacatcaagtgtatcatatgccaagtacgccccctattgacgtcaatgacggtaaatggcccgcctggcattatgcccagtacatgaccttatgggactttcctacttggcagtacatctacgtattagtcatcgctattaccatggtgatgcggttttggcagtacatcaatgggcgtggatagcggtttgactcacggggatttccaagtctccaccccattgacgtcaatgggagtttgttttggcaccaaaatcaacgggactttccaaaatgtcgtaacaactccgccccattgacgcaaatgggcggtaggcgtgtacggtgggaggtctatataagcagagctcgtttagtgaaccgtcagatcgcctggagacgccatccacgctgttttgacctccatagaagacaccgggaccgatccagcctccgggatccagatcttctagaaagcttggtaccgatatcatggaactgggcctgcggtgggtgtttctggtggccatcctggaaggcgtgcagtgccacggcgagggcaccttcaccagcgatgtctcctcttacctggaagagcaggccgctaaagagttcatcgcctggctggtgaagggaggaggcggcggcggaggctctggcggaggcggctccggcggcggtggctccgctgagtccaaatacggccctccatgtcctccttgccctgctcctgaggctgctggcggaccctccgtgttcctgttccctcccaagcccaaggacaccctgatgatcagccggacccctgaagtgacctgtgtggtcgtggacgtgtctcaagaggaccctgaggtgcagtttaactggtacgtggatggcgtggaagtacataacgccaagaccaagcctcgggaggaacagttcaactccacctacagagtggtgtctgtgctgacagtgctccaccaggactggctgaacggcaaagagtacaagtgcaaggtctccaacaagggcctgccttcctccatcgagaagaccatctctaaggccaagggccagcctagagagcctcaagtgtacaccctgcctccctctcaggaagagatgaccaagaatcaggtgagcctgacctgcctggtcaagggcttctacccttctgatatcgccgtggaatgggagtctaatggccagcccgagaacaactacaaaaccacaccacctgtgctggactccgacggctccttcttcctgtactccagactgaccgtggacaagtctagatggcaggagggcaacgtgttctcctgctccgtgatgcacgaggccctgcacaaccactatacacagaagtccttgagcctgtctctgg

SEQ ID NO: 15 - DNA, 19 bp, synthetic construct
  source 1..19: mol_type = other DNA
tgcagccacactaagatgg

SEQ ID NO: 16 - DNA, 20 bp, synthetic construct
  source 1..20: mol_type = other DNA
ccagagacaggctcaaggac

SEQ ID NO: 17 - DNA, 96 bp, synthetic construct
  source 1..96: mol_type = other DNA
gatagtcacccacaccagaggttttagagctagaaatagcaagttaaaataaggctagtccgttatcaacttgaaaaagtggcaccgagtcggtgc

SEQ ID NO: 18 - DNA, 9126 bp, synthetic construct
  source 1..9126: mol_type = other DNA
gtaagtaaagcagcagatgagggcccagtgtggctgtggggcagctccttatgcagcgtgctggcagttttttactgtgattaaaggagatcctgggcttagagcctgtggtggtagtcttgcctctcaacaacacatctgtgtcctgttctgttgtgactgctttctagaactgttggattgtatggccacattgtaactgaggaatactacattgtaatatctcagattttcctctctaaatcataaataaagtagaaatttcaccaaagtgaattcatgtttatactacaaaagtaacagcatggctactctgataacagagtgactagatttgtatgtaataactagaactggctataaatgatttgttttggagatgcctgtgagaatgtgctttattaatttagtgaatagttaatagataatagcgggtagttcttatcattcaggccagagaacacaaatgagaccagattagctggaagttgtcacattcatattcagatactatggatgaagtaatgcctttcagggtatcttggaactgtaaagcatttttaaaattgtagtagtgaatttgaatgaaaggcctaaaggtagtgagtggtaaacattattcgggaactagtgcaagttaatttgaaaaaaacaggtcactgcagttcctgtgctgaggactccatgtcaggtactaccaagcagaaataggcttaatttctggaggaaatattttccttttttgttgtagtggaggtttgaaattacatacaacttgtatagatgacttattcatgacatttggcttttcctttataactcaagggcggaatgcctacctagcctacatgagagtttgaactctagtattgcaaataaatgaatgacttataaataagtatcttagagctatgaatatcttagagaaaccatcattcctcacgtcacagtggacacggtaatgtttgaagcatctccaacatctgtttggtctgtacttgaatacttccagaatggtaagagcacaggctttcatagctcagtccagtacatttgttggcctgctctgattgctaggaagcttttgcttgtatgagacgcaagcctgtccttgtgtgatgctgctcccagcctccagttctgtctccccgagagcctgcttccgtgggacaacctgcacatctttaaaggtcctgtcatgctcttcggtacaagctagccacctacactcaaatacttttctgatggcacctccccacccccaccccagtctctcatcagtctggttgcctttaattgaaggaattccagtttttcaaagtccttttaaaatccagagttgagcataatctcacaagagtgagtcagcagtgccagttgtgtggtgcttatctatgtcttcatctggacactgtactataatggccgtgccatctgtgctttattatcaacatctcaccgtttgcttgtacttggaaacctctagaatagtggttctcaaccaggcacagttttgccccccaggagacatttggttgtcacactggggaagtgctaactggaatcttgtaggtaggggtaatgatgctgttagatactttataatgtacaggacagcctccgacaacaaatcattaacccccgatgtctccagggcttggatggaggaaccctgttctgcattatcatgaatgcagctgtcaagttttgttctggtgaaggtagccaggcttgtaagcctttggagtgtctccatactggaattttcttgatggtttcaacccagtatgtgagcttgtattaggggttcatctgtcttcaacagaatattatttgttgttgctgctgttgtttttgagatgttcccatgtaacccaagctggcctccaacttgctatgtgaagttaaagttgaccttgaactccagctctcctgccttcccctttccagtgctaggatgacaagcatgcacctggcctcacaaacatttgccaagcaaggtgctgtgattgcagatggtgatttgcaaaatagaggtagaaatacctgatggcagtaatgtgagcattggggataaagtgtaagtgtgaagggtaccagtgctgtgtttgggagcacaaggagctcacttgtgtgcttaggcgagccttcaaggtagtcttaaaaagtgtattcagtttatgagaaaagcagggcaggagaatttctgagacatgggcacaaagtgaacaaagagagggaggtagaaagcagaggccccttcccctctttagggagtggccagccatccttctaaaattagtgtgttttgttttctcttttgaaacagacttgtgcagcccaagctttcctcaaagtggtgatcctcctgcctctctagtgctaggattacaggcatataccacacgtgaccagtacattttctgtatagggctaaatagtaaatgttcttttccttacagactatgtagtctctgttaacagtcagttgtagaccatgcacatatgggctgggggtagagcttagactggatcacatgccacaaggccctgggttctattcccagaaccacagcacaggaaaaaggatagcatgtaaatgagcatgctggccagaattgacttaggggctgtagtgagcgtctcggtccttggactaaaatcccgggagtagcaggagatggggatagaaagatagcaaagatccagatctagaacatagtgatagctccacgagtgtttgtgatgtttacgaagagtaggagacttgcagatctgggagccaggagtaatgtggctagaggagcgtatagatgtggcgcacgcctttgatcccagcactcgggaggcaggggggtgggtctctgtgagtttgaggccagcctggtctacagagttccaggacagtcagaactatatagtgagaccctgtctcaaaacaaacaaacaaaaacaaaacaaaagaggagcattttagaagggatattctggcagcagcaggtagccaggaaacaaaggaaagaagggacgctatggcctgctagaagacacttgagtttcatttaacagttgaaggggagaatctaagacccaaggagctttgtctgctgttggaatttgcataatgagccctgagttgaatgtgagtcaaaggttttgaatcacattcattgaaaagatttgtttaggctaggtggtggtggtgcacacctttaatcccatcacctgggaggcagaggcaggtggatctctgagttcaaggccagcctggtttacagatggagttccaggacatccagggctacacagagaaaccctgtctcgaaatccccccccaccaccaccaccaaaaaaagggaaaaacaaaacaaaacagaaaaaagcttcgtctaggtctgggcatggtggttgcacacctttcatgccagcactctggaggcagagtcaagtggatctgagttcaaggcccactagggctatccagtaagatccttcctcaaaacaaaagataggtttttctcaatgccttgagttgctgctggttgatgaatggtaaatatttagtagttgagagtctatcacgatgtgtcattcagtcgtgttcagactgcatgttgaagacaaagtggctagctctgccttctacccactacctccccactctaaatggtgagtctgttaacaagaattggcacaagagcaaagttggtggggaagtgagtacatttggttggtgcgtactgaatgtagtccttgggcgtaaggagcataagttgaaacccactggaaatgtgggtctgaggtcaagcaaatgacacagatcctagatgccttcagggtggccacacaaacaaggaagaagatagggactggagagagaaagggagccagagaaaaagacagtagtcaggagaggtgggtcaggaaggctgacttcctgtatggcctggaagagggagtagggaggagctggagaaaacactagttcttgtctcttgtactcaacattttgaaaatgttttcagttgagccctgggcacagagtgtgtgaggtagaagtaagctgggatgagagagcaggaagcagaagtgtggagttttgttttgtttttaaagtttgatacttggaagaaaaaccattgaggcagtagtagtagctcaggggcattgaaactttgaagtttagaaagttagagctgggcatggtgattcatgcctttcagtcccagcgctggggaaggagaggcagatggagttctaggccagctagggctacgtagtaagaacccatttctaaattaatttcattaaagcctcaaaagttttggcatagtttaggccctagctttaggccagcctcagttaatgattactgtatgagtgttcatgagcaaatgtttgagaaatgttaagtaaaatcaaactgtttcagaacttatcaggcgggaccttttggcttgctaataactaagagaagtattttctaaattctgtaagcttatgttataaaccattttccagacattagctgagcatggtttgggaaatgctgatctaagcagaagagaagataggagggtggatgggattatgcaatctgatattagctgtcactttcttgctttgtactccttaccaattagttgcttctgtttgcaagcctggcttgccccattcgtttcttggggccatttaatcgtgaacagggtcaaggatgtacgagctcttcatccagtgtactatgggtttatctcataggctcttccttctctcttcagtttttctatcctatatgtaacatctgtgtagaagagtctatatgctagacttatttattttctgaattggattttaacagcagccgatgctggcctcagactcacagcagtctgttgaagtctgagattagaaacgggggccactgccctggtcttaaactggtattaggctcagtaggtttggggcctcgatggggatcaggaagaagtagccacagccctgtcttcggaggccagacagacattcaggaggcttgccttacctcagtcagtgattgacagtggttctattttggcttacaaatccacttagttggcctgaggaggccagtgtttacagatgataacagctgcatgatctttaaccatccttgtcccgggagcctgttttaagcatggctgtttttgctgcatggcattcacaggtactgctcttgagaaatgcaatcctttgataactaagtcttcttggcttcctaagcagcttagtttctgagtcagatgttagcctgattttcctgtttaccccgggttgtacctttgtttcctttagtgtgcagttggcttactgatcactttcttcctcctcctcctcctcctcctcctcctcctcctcttcttcttcctcctcctcctcctcctcctcctcctcctcctcctcctcctcctcctcctcctcctcctcctcctcctcctcctcctcctcctcctcctcctcctcctcctcctcctcctcctcctcctcctcctcctcctcctcctcctcctcctcctcctcctcctcctcttcttcttcttcttcttcttcttcttcttcttcttcttcttcttcctattattttcatcatgcttatcttacgcaaaaacaagccaaccaggaccttgccacacacactgtctcaccctaccacagacttctgggcatcctggctcttagttcacatttcaggttctcatcctaactttactgctttttccctgtggattggtagctttgagagcttctgtcaaaacactgtcattctgcatcccatatactcaaaggcctcctaaatagtcggcagatatgaagaaaccaagggtccaaggatattgttcatggtaccctaaatatcccagagcattgattgggaaagaatggctttccttgcaagaagcaggtgcagtggtctttgaattttgctcttggagtattggattactgtcagtggccttctgaaaggaggggatgggttctttctctttcctattcctctttttttattttatatttaattttttttaaaattttttgagacagggtttctgtgtagtcctggccgacctggagctcactgtgttgaccaggttggcctcaaacctctttgcctctgcctcccaagtaccaaaggcatatgccatcacaactagctgaatttatttagcctgacagattttaagtaagaataaaggggttagaatggggtggcttgtgcctataatgccagcatcttggaaggctaaagcagaagcttgccgtgagtttcaggcattctgggctacatggtactttgcaggccagcctgggttacaatgagaaatctgtctcaggaaaacaaaagggagcaaacagaagtaagggggatttgactccagtgttcagagccttttttcagttttcctttattttaggaagactgatcgaagcctggtggtggtggcacactcctttagtcccagcactctggaggtagaggcaggcagatctctgtgagttctagaccagcctggtctacaagagctagttctaggacagcctccaaagccacaaagaaaccctgtctcaaaaaaacaaaacaaaacaaaacaaaaagactgattgcagtcctgttcctcagtgggaatcctcggggagtggagctatgcgctcagacacaccagggtgtttaactgtgctggagtggatccacccaccttccactctgcacgccacgattacatttcttcacagatccctgttcagctcccacgggattgccattcagaactaggaccgatgagcctgtcactgcttgaaagtgtagtgttgagcatctgctcatttccctccaaggtctgacgtaactttggtcagatgctctgttagttctcagaaccctctggtgcttggcgagcagtagggaaatgctggtggctctgtatggctctgttggaggctagagtagggtgtgctttccctgtgccaccacgtgaagccgatttatcaacgtgtctcctccatgagggcatatgtgatacttgtccctgtctcatcactgaggccctctggcctggcagaggaacctggctggttttaggcacacactgtgttttaaagttgttaccgtgggagctctgggtcttcagttgatgttttctgtggactgtaataggttctcctgacattttgttcttgtaagagtgggagaatatacttgaattttagttctctccccttatttaaatccagcttattccaaaaactgtttcttcttcgaaagatgatttcagccttggtctcttcttttttgttgtagtgtatacttgctatgtggcccaggcaagctgctctctgtcctcttttgtaatatggaaataaaaatatcctgctgcattctgtgatgatgcagtgagatttatgtaatataaaagtgtacctcagtgtgcctcagatgctgggcacagcagccgttcagtcacatgttctcttgcttttttttcccctcacagacccctgttcctaaaggttcagaggtcatgtctagttttagaaaggttaaaactgtcaaggcttttatgttagggactgatttgggaagcatgttctccttgagacaggctgtaaattgtggttggaagcggaagtgctagtgcacactggggaggccgaggcagggggatctgtacatttcaaggctgtctagtctacatagttcaaggctagtctgagattctgtctttaaaagttggggaaatgtgattggattccaggagagcccgcagaaatcttagtcccagcctacttagctgaactttcctgtgaacatcattgtaactgggaggggttgttgtgtattgtttgttttgtttggggggagctagggaattgagcccagggccaccagatgatgctaggccagggctctgccactaagctacatcttcagtcatctttttttttttttttttttttttttttttttttttttttttgtttttttgagacagggtttctctggctttggaggctgtcctggtattagctcttgtagaccagattggtctcgaactcacagagatctgcctgcctttgcctcctgagtgctgggattaaagtcgtgtgccaccaacgcccggtttatttttgtttttttaatttatttatttatatgtatgagtattttgcctgcatttatgtctgtggcccatttgtgtgccgggcatctgtggaggcagaaaacacctgatcccctgtaactagaggtgcagcctgttgaaaaccactgtataggtgctaagaattgaatctgggtcctctggaagagcagccagtcctcctaatcacttaacattctctctagctcctcttaaaaacaaaaacaaagacaaaaaacaccctttttgttttgaaataggttctccctaagttgttcagggtggctttgaactcaatctgtggtatggggatcattgtactgggattacttttctatatcttcctgggtaactgagaccatcaacctgagtcattagaccacagttttaaccatgttataaaatgagggcatttgtggttcccaaacaaaggttggtgaacactagtccttgccacaggtaatcttttgtttgtttgtttgtttgtttgtttttgagacatggtttctctgtggctttggaggctgtcctggaactaactcttgtagaccaggctggtttggaactcacagagatcctcctgcctctgcctcctgaatgctgggactaaaggcatgcaccaccatcttttgccctcattggtgtcttgtaattcccttggtaccaggccactgaaagttactttcatggtggacatatggggcaccaatatcctccagctaaaagtgaaggctttaatataattttatatttcatctttttaacaatcataaaacaaacagttagtccccattttacagagataaaaaaatgaaagcatagaaacatctagctgtcggtcccagtgcctggaggtagagacaggtgaatcctaagggttctctggctgtagagtctgagagctccagattcagtgagagaccctgtctcagaaaataacatggaggcctggtgt

SEQ ID NO: 19 - DNA, 2113 bp, synthetic construct
  source 1..2113: mol_type = other DNA
gtggttgcacacctttcatgccagcactctggaggcagagtcaagtggatctgagttcaaggcccactagggctatccagtaagatccttcctcaaaacaaaagataggtttttctcaatgccttgagttgtgactggtgagtactcaaccaagtcattctgagaatagtgtatgcggcgaccgagttgctcttgcccggcgtcaatacgggataataccgcgccacatagcagaactttaaaagtgctcatcattggaaaacgttcttcggggcgaaaactctcaaggatcttaccgctgttgagatccagttcgatgtaacccactcgtgcacccaactgatcttcagcatcttttactttcaccagcgtttctgggtgagcaaaaacaggaaggcaaaatgccgcaaaaaagggaataagggcgacacggaaatgttgaatactcatactcttcctttttcaatattattgaagcatttatcagggttattgtctcatgagcggatacatatttgaatgtatttagaaaaataaacaaataggggttccgcgcacatttccccgaaaagtgccacctgacgtcgacggatcgggagatctcccgatcccctatggtgcactctcagtacaatctgctctgatgccgcatagttaagccagtatctgctccctgcttgtgtgttggaggtcgctgagtagtgcgcgagcaaaatttaagctacaacaaggcaaggcttgaccgacaattgcatgaagaatctgcttagggttaggcgttttgcgctgcttcgcgatgtaggtttgtctggtcaaccaccgcggtctccgtcgtcaggatcatgacattgattattgactagttattaatagtaatcaattacggggtcattagttcatagcccatatatggagttccgcgttacataacttacggtaaatggcccgcctggctgaccgcccaacgacccccgcccattgacgtcaataatgacgtatgttcccatagtaacgccaatagggactttccattgacgtcaatgggtggagtatttacggtaaactgcccacttggcagtacatcaagtgtatcatatgccaagtacgcccctatgacgtcaatgacggtaaatggcccgctggcattatgcccagtacatgacctttatgggactttcctacttggcagtacatctacgtattagtcatcgctattaccatggtgatgcggttttggcagtacatcaatgggcgtggatagcggtttgactcacggggatttccaagtctccaccccattgacgtcaatgggagtttgttttggcaccaaaatcaacgggactttccaaaatgtcgtaacaactccgccccattgacgcaaatgggcggtaggcgtgtacggtgggaggtctatataagcagagctcgtttagtgaaccgtcagatcgcctggagacgccatccacgctgttttgacctccatagaagacaccgggaccgatccagcctccgggatccgccaccatggaactaggtctacgatgggtgtttctagtggccatcctggaaggcgtgcagtgtgctcctcccagactgatctgcgactcccgcgtgctggaacggtacctgctggaagccaaagaggctgaaaacatcacaacaggctgcgccgagcactgcagcctgaacgagaatattaccgtgcctgacaccaaggtgaacttctacgcctggaagcggatggaagtgggtcagcaggccgtcgaagtgtggcagggcctggccctgctgtctgaagctgtcctccggggccaagctctgctcgtgaactcctctcagccttgggaacccctgcaactgcacgtggataaggccgtgtctggcctgagatctctgaccacactgctgcgggctttgggcgcccagaaagaggctatcagcccccctgatgctgcttccgccgcccctctgagaacaatcaccgccgataccttccggaagctttttagggtttacagcaatttcctgcggggcaagctgaagctgtataccggcgaggcctgcagaaccggcgacagaggctccgagagaaaatgttgcgtggagtgtcctc

SEQ ID NO: 20 - DNA, 20 bp, synthetic construct
  source 1..20: mol_type = other DNA
gtctgggcatggtggttgca

SEQ ID NO: 21 - DNA, 19 bp, synthetic construct
  source 1..19: mol_type = other DNA
gaggacactccacgcaaca

SEQ ID NO: 22 - DNA, 3121 bp, synthetic construct
  source 1..3121: mol_type = other DNA
gagtcagtggatctgagttcaaggcccactagggctatccagtaagatccttcctcaaaacaaaagataggtttttctcaatgccttgagttgtgactggtgagtactcaaccaagtcattctgagaatagtgtatgcggcgaccgagttgctcttgcccggcgtcaatacgggataataccgcgccacatagcagaactttaaaagtgctcatcattggaaaacgttcttcggggcgaaaactctcaaggatcttaccgctgttgagatccagttcgatgtaacccactcgtgcacccaactgatcttcagcatcttttactttcaccagcgtttctgggtgagcaaaaacaggaaggcaaaatgccgcaaaaaagggaataagggcgacccggaaatgttgaatactcatactcttcctttttcaatattattgaagcatttatcagggttattgtctcatgagcggatacatatttgaatgtatttagaaaaataaacaaataggggttccgcgcacatttccccgaaaagtgccacctgacgtcgacggatcgggagatctcccgatcccctatggtgcactctcagtacaatctgctctgatgccgcatagttaagccagtatctgctccctgcttgtgtgttggaggtcgctgagtagtgcgcgagcaaaatttaagctacaacaaggcaaggcttgaccgacaattgcatgaagaatctgcttagggttaggcgttttgcgctgcttcgcgatgtaggtttgtctggtcaaccaccgcggtctccgtcgtcaggatcatgcggccgccatatcataatatgtacatttatattggctcatgtccaacattaccgccatgttgacattgattattgactagttattaatagtaatcaattacggggtcattagttcatagcccatatatggagttccgcgttacataacttacggtaaatggcccgcctggctgaccgcccaacgacccccgcccattgacgtcaataatgacgtatgttcccatagtaacgccaatagggactttccattgacgtcaatgggtggagtatttacggtaaactgcccacttggcagtacatcaagtgtatcatatgccaagtacgccccctattgacgtcaatgacggtaaatggcccgcctggcattatgcccagtacatgaccttatgggactttcctacttggcagtacatctacgtattagtcatcgctattaccatggtgatgcggttttggcagtacatcaatgggcgtggatagcggtttgactcacggggatttccaagtctccaccccattgacgtcaatgggagtttgttttggcaccaaaatcaacgggactttccaaaatgtcgtaacaactccgccccattgacgcaaatgggcggtaggcgtgtacggtgggaggtctatataagcagagctcgtttagtgaaccgtcagatcgcctggagacgccatccacgctgttttgacctccatagaagacaccgggaccgatccagcctccgcggccgggaacggtgcattggaacgcggattccccgtgccaagagtgacgtaagtaccgcctatagagtctataggcccacccccttggcttcttatgcatgctatactgtttttggcttggggtctatacacccccgcttcctcatgttataggtgatggtatagcttagcctataggtgtgggttattgaccattattgaccactcccctattggtgacgatactttccattactaatccataacatggctctttgccacaactctctttattggctatatgccaatacactgtccttcagagactgacacggactctgtatttttacaggatggggtctcatttattatttacaaattcacatatacaacaccaccgtccccagtgcccgcagtttttattaaacataacgtgggatctccacgcgaatctcgggtacgtgttccggacatgggctcttctccggtagcggcggagcttctacatccgagccctgctcccatgcctccagcgactcatggtcgctcggcagctccttgctcctaacagtggaggccagacttaggcacagcacgatgcccaccaccaccagtgtgccgcacaaggccgtggcggtagggtatgtgtctgaaaatgagctcggggagcgggcttgcaccgctgacgcatttggaagacttaaggcagcggcagaagaagatgcaggcagctgagttgttgtgttctgataagagtcagaggtaactcccgttgcggtgctgttaacggtggagggcagtgtagtctgagcagtactcgttgctgccgcgcgcgccaccagacataatagctgacagactaacagactgttcctttccatgggtcttttctgcagtcaccgtccttgacacgaagcttgccgccaccatggacatgagagtgcctgctcagctgctgggcctgctcctgctgtggctgagaggcgctagatgtgatatcgtgatgacacagtccccactttctctgcctgtcacccctggcgaacctgcttctatctcttgccggtcctcccagagcctcctgtattccatcggctacaactacctggattggtacctgcagaagagcggccaatcccctcagctgctgatctacctgggctccaaccgggccagcggagtgcccgatagattctccggctccggatctggcaccgacttcacactgaagatcagcagagtggaagctgaggacgtgggcttttactactgcatgcaggctctgcagaccccctacaccttcggccagggaaccaagctggaaatcaagcggaccgtggccgctccttctgtgttcatctttcctccttccgacgagcagctgaaatctggcaccgcctccgttgtgtgcctgctgaacaacttctaccctagagaggccaaggtgcagtggaaggtcgacaacgccctgcagtctggcaactctcaagagtccgtgacagaacaggactctaaggactccacctactccctgtcctctaccctgaccctgtccaaggccgactacgagaagcacaaagtgtacgcctgcgaggtgacccac

SEQ ID NO: 23 - DNA, 19 bp, synthetic construct
  source 1..19: mol_type = other DNA
actcgcctctattgaagct

SEQ ID NO: 24 - DNA, 1191 bp, synthetic construct
  source 1..1191: mol_type = other DNA
gctcctcccagactgatctgcgactcccgcgtgctggaacggtacctgctggaagccaaagaggctgaaaacatcacaacaggctgcgccgagcactgcagcctgaacgagaatattaccgtgcctgacaccaaggtgaacttctacgcctggaagcggatggaagtgggtcagcaggccgtcgaagtgtggcagggcctggccctgctgtctgaagctgtcctccggggccaagctctgctcgtgaactcctctcagccttgggaacccctgcaactgcacgtggataaggccgtgtctggcctgagatctctgaccacactgctgcgggctttgggcgcccagaaagaggctatcagcccccctgatgctgcttccgccgcccctctgagaacaatcaccgccgataccttccggaagctttttagggtttacagcaatttcctgcggggcaagctgaagctgtataccggcgaggcctgcagaaccggcgacagaggctccgagagaaaatgttgcgtggagtgtcctccttgccccgccccacctgtggctggaccttccgtgtttctgttccctcctaagcccaaggacaccctgatgatctccagaacccccgaagtgacctgtgtggtcgtggacgtgtcacacgaggaccctgaggtgcagttcaactggtacgtggatggcgtcgaggtgcacaacgccaagaccaagcctagagaagagcagttcaactccaccttcagagtggtgtctgtcctcacagtggtgcaccaggactggctgaatggcaaagagtacaagtgcaaggtgtccaacaagggcctgcctgctccaatcgagaagaccatctccaagaccaagggccagccacgggagcctcaggtgtacaccctgcctccctctcgggaggagatgaccaagaaccaggtctccctgacctgcctggtgaagggcttttacccttctgacatcgccgtggaatgggagtccaacggccaacccgagaacaactacaaaaccacccctcctatgctggactccgacggctctttcttcctgtactccaagctgactgtggacaagtctagatggcagcagggaaacgtgttctcttgctccgtgatgcatgaggccctgcataaccactacacccagaagtctctgtccctgagccctggaaagtga

SEQ ID NO: 25 - DNA, 645 bp, synthetic construct
  source 1..645: mol_type = other DNA
gacattcagatgactcagagcccctcctccatgtccgcctctgtgggcgacagggtcaccttcacatgccgcgctagccaggatatcaacacctacctgagctggtttcagcagaagccagggaaaagccccaagacactgatctaccgggctaatagactggtgtctggagtcccaagtcggttcagtggctcagggagcggacaggactacactctgaccatcagctccctgcagcctgaggacatggcaacctactattgcctgcagtatgatgagttcccactgacctttggcgccgggacaaaactggagctgaagcgtacggtggctgcaccatctgtcttcatcttcccgccatctgatgagcagttgaaatctggaactgcctctgttgtgtgcctgctgaataacttctatcccagagaggccaaagtacagtggaaggtggataacgccctccaatcgggtaactcccaggagagtgtcacagagcaggacagcaaggacagcacctacagcctcagcagcaccctgacgctgagcaaagcagactacgagaaacacaaagtctacgcctgcgaagtcacccatcagggcctgagttcgcccgtcacaaagagcttcaacaggggagagtgttga

SEQ ID NO: 26 - DNA, 2142 bp, synthetic construct
  source 1..2142: mol_type = other DNA
gaagtgcagctggtcgagtctgggggagggctggtgcagcccggcgggtcactgcgactgagctgcgcagcttccggattcgcctttagctcctacgacatgtcctgggtgcgacaggcaccaggaaagggactggattgggtcgctactatctcaggaggcgggagatacacctactatcctgacagcgtcaagggccggttcacaatctctagagataacagtaagaacaatctgtatctgcagatgaacagcctgagggctgaggacaccgcactgtactattgtgccaaccgctacggggaagcatggtttgcctattgggggcagggaaccctggtgacagtctctagtgctagcaccaagggcccatcggtcttccccctggcaccctcctccaagagcacctctgggggcacagcggccctgggctgcctggtcaaggactacttccccgaaccggtgacggtgtcgtggaactcaggcgccctgaccagcggcgtgcacaccttcccggctgtcctacagtcctcaggactctactccctcagcagcgtggtgaccgtgccctccagcagcttgggcacccagacctacatctgcaacgtgaatcacaagcccagcaacaccaaggtggacaagaaagttgagcccaaatcttgtgacaaaactcacacatgcccaccgtgcccagcacctgaagccgcaggggctccgtcagtcttcctcttccccccaaaacccaaggacaccctcatgatctcccggacccccgaggtcacatgcgtggtggtggacgtgagccacgaagaccctgaggtcaagttcaactggtacgtggacggcgtggaggtgcataatgccaagacaaagccgcgggaggagcagtacaacagcacgtaccgtgtggtcagcgtcctcaccgtcctgcaccaggactggctgaatggcaaggagtacaagtgcaaggtctccaacaaagccctcccagcccccatcgagaaaaccatctccaaagccaaagggcagccccgagaaccacaggtgtacaccctgcccccatcccgggatgagcttaccaagaaccaggtcagcctgacctgcctggtcaaaggcttctatcccagcgacatcgccgtggagtgggagagcaatgggcagccggagaacaactacaagaccacgcctcccgtgctggactccgacggctccttcttcctctacagcaagctcaccgtggacaagagcaggtggcagcaggggaacgtcttctcatgctccgtgatgcatgaggctctgcacaaccactacacgcagaagagcctctccctgtctccgggtaaaggtggcggagggtctggtggtggaggatcagggggtggaggttcaggaggcgggggaagtcaggtgcagctggtcgagtctggggccgaagtgaagaaacccggcgcctcagtgaaggtcagctgcaaggccagcgggtacagtttcactggatataccatgaactgggtccgacaggcccctggccagtgtctggagtggatcggcctgattaacccttacaacaacatcactaactacgcacagaagttccaggggagagtgacctttacagtggacaccagcatttccacagcctacatggaactgtcccggctgagatctgacgatacaggcgtgtacttctgcgctaggctggattaccgcagctattggggacagggcacactggtgactgtcagcgcaggagggggtggaagtggcggaggtggttctggaggtggtgggtctggtggaggcggttcacaggctgtcgtcactcaggaaccttcactgaccgtgtctcctggcgggactgtcaccctgacatgcggcagctccacaggggccgtgaccacaagtaacttcccaaattgggtccagcagaagccaggacaggctccccggagtctgatcggaggcaccaacaacaaggccagctggacacccgcacggttcagcggcagcctgctgggcggcaaggccgctctgacaattagcggagcccagcctgaggacgaagccgagtactattgcgctctgtggtactccaaccactgggtgttcggctgcggcaccaagctgactgtgctgcggtga

SEQ ID NO: 27 - DNA, 642 bp, synthetic construct
  source 1..642: mol_type = other DNA
caaccaggtctaactcaaccaccaagtgtgtctgtcgccccaggacaaaccgccagaatcacctgtggcggcaacaacatcggctctaagtccgtccattggtatcagcagaagcctggtcaggcccccgtgctcgtggtgtacgacgactccgaccggcctagcggcatccccgagcggttctccggctccaactccggcaataccgctaccctgaccatctccagagtggaagctggcgatgaggccgattactactgccaggtgtgggactctagctctgatcactacgtgttcggcaccggcaccaaagtgaccgtgctgtcctccgcctctacaaagggcccatctgtttttcctctggctccttcctccaagtctacctctggcggaacagctgctctgggctgcctggtgaaggactacttccctgagcctgtgactgtgtcctggaacagcggagccctgacctccggcgtgcacaccttccctgccgtgctgcagtcctctggcctgtactccctgtcttccgtggtcaccgtgccttcttctagcctgggcacccagacctacatctgcaacgtgaaccacaagcccagcaacacaaaagtggacaagaaggtggaacctaagtcctgctaa

SEQ ID NO: 28 - DNA, 1392 bp, synthetic construct
  source 1..1392: mol_type = other DNA
caagtgcaactagtgcaaagtggtgcagaagtgaagaagcctggcgcttctgtcaaggtttcttgcaaggccagcggctacaccttcaccggctattacatgcactgggtcagacaggcccccgggcagggcctggaatggatgggctggatcaaccctaactccggaggcacaaattacgctcagaagtttcagggcagagtgaccatgacccgggatacctccatctccacagcttacatggaactgagcaggctgagatccgacgacaccgctgtgtactactgcgccagatcccccaatccttactactacgactcctccggctactactacccaggcgccttcgacatctggggacaaggcaccatggtcaccgtgagctctgcctccgtggccgctccgtccgtgttcatcttccccccctctgacgagcaactgaagtccggcaccgcttccgtcgtctgtctgctgaacaacttctatcctcgggaggccaaagtgcagtggaaggtggacaacgctctgcagtctggcaattctcaagagtctgtgaccgagcaggatagcaaggactccacctactccctctctagcaccctgaccctgtccaaagccgactacgagaagcacaaggtgtacgcctgcgaggtgacccaccagggactgtcctctcctgtgacaaaatcttttaaccggggagagtgcgacaagacccacacctgccctccttgtcctgctcccgagttgctgggcggccctagtgtgtttctgttccctcctaagcccaaggatacactgatgatctctcggaccccagaagtgacctgtgtggtggtggacgtgtcccacgaggaccctgaggtgaagttcaactggtacgtggatggcgtggaagtgcacaacgccaaaaccaagcctcgggaagagcagtataacagcacatacagagtggtgtccgtgctgaccgtgctgcatcaggactggctgaacggcaaagagtacaagtgcaaggtgagcaacaaggccctgcccgcccctatcgagaagaccatctccaaggctaagggccagcctcgcgaacctcaggtgtgcacactgcctccttcaagagacgagctgaccaagaaccaggtgtctctgtcttgtgccgtgaaaggcttctacccttccgatatcgccgttgagtgggagtccaacggacagcctgaaaacaactacaagaccacccctccagtgctggactccgacggctctttcttcctcgtgtctaagctgaccgtggataagtccagatggcagcagggcaacgtgttctcttgctccgtgatgcatgaagctctgcacaaccactacacacagaaatctctgtccctgtctccaggcaagtaa

SEQ ID NO: 29 - DNA, 645 bp, synthetic construct
  source 1..645: mol_type = other DNA
gatatccaaatgactcaaagtccaagtagtctctccgccagcgtcggcgacagagtgacaatcacctgttctgcttctcaggacatctccaactacctgaattggtatcagcagaagcctggcaaggcccctaaggtgctgatctacttcacctcctctctgcactctggcgtgccctcccggttctccggctctggatctggcaccgattttaccctgaccatcagcagcctgcagcctgaagattttgctacctactactgccagcagtactctaccgtgccttggaccttcggccagggaacaaaagtcgagatcaagcggactgtggccgctccttctgtgttcatcttccctccatccgacgagcagctgaagtctggcaccgccagcgtggtgtgcctgctgaacaacttctaccccagagaggccaaggtgcagtggaaggtggacaacgccctgcagtccggcaactcccaagagtccgttaccgaacaggattccaaggactccacctattccctgtcttccaccctgacactgtccaaagctgactacgagaagcacaaggtgtacgcctgcgaagtgacccatcaaggcctgtctagccctgtgaccaagtccttcaacagaggcgagtgctaa

SEQ ID NO: 30 - DNA, 1362 bp, synthetic construct
  source 1..1362: mol_type = other DNA
gaagtgcaactagtggaaagtggtggtggtctcgtgcagcctggcggcagcctgagactgtcttgtgccgcttctggctacaccttcaccaactacggcatgaactgggtgcggcaggctcccggcaagggactggaatgggtcggctggatcaacacctataccggcgagcccacctacgccgccgacttcaagcggcggttcacattcagcctggatacctccaagtctacagcctacctgcagatgaatagcctgagagccgaggacaccgctgtgtactactgcgctaagtaccctcactactacggcagctcccactggtatttcgacgtgtggggccagggcaccctggtcacagtctcttctgcctccaccaaaggcccttccgtgttccctctggccccatcatctaaatctacctccggcggcaccgctgccctgggctgtctggtgaaggactacttcccagaacctgtgaccgtgtcctggaactccggcgctctgacttctggcgtgcacacctttcctgccgtgctgcagtcctctggtctatactctctgtcctccgtggtgacagtgccttccagctctctgggaacacagacctacatctgtaacgtgaaccacaagccctccaacacaaaggtggataagaaggtcgaacccaagtcctgtgacaagacccacacctgccctccttgccctgctcctgaactgctgggaggcccttccgtgtttctgtttcctcctaagcccaaagatacactgatgatcagccgcaccccagaagtgacctgcgtggtcgtggacgtgtctcacgaggaccctgaggtgaagttcaactggtacgtggatggcgtggaagtgcacaacgccaagaccaagcctagagaggaacagtacaactccacctacagagtggtgtccgtgctgaccgtgctgcatcaggactggctgaacggcaaagagtacaagtgcaaggtgtctaacaaggccctgcccgctcctatcgagaagaccatctctaaagctaagggacaacctcgggagcctcaagtgtataccctgcctccctgcagagacgagctgaccaagaaccaggtgtccctgtggtgcctggtgaagggcttctaccccagcgacatcgccgtcgagtgggagtccaatggccagcctgagaacaactacaaaaccacccctccagtcctggactctgacggctctttcttcctgtactccaagctgaccgtggacaagtccagatggcagcagggcaacgttttctcctgctctgtgatgcacgaggccctgcacaatcattacacccagaagtccctgtccctctctcctggcaagtaa

SEQ ID NO: 31 - DNA, 2713 bp, synthetic construct
  source 1..2713: mol_type = other DNA
ctcgacgccatccacgtaccagttgaactgcacctcagggtcctcgtgtgacacgtccacgaccacacaggtcacttcgggggttctggagatcatcagggtgtccttgggcttaggagggaacagaaacacggaaggtccagccacaggtggggcggggcaaggaggacactccacgcaacattttctctcggagcctctgtcgccggttctgcaggcctcgccggtatacagcttcagcttgccccgcaggaaattgctgtaaaccctaaaaagcttccggaaggtatcggcggtgattgttctcagaggggcggcggaagcagcatcaggggggctgatagcctctttctgggcgcccaaagcccgcagcagtgtggtcagagatctcaggccagacacggccttatccacgtgcagttgcaggggttcccaaggctgagaggagttcacgagcagagcttggccccggaggacagcttcagacagcagggccaggccctgccacacttcgacggcctgctgacccacttccatccgcttccaggcgtagaagttcaccttggtgtcaggcacggtaatattctcgttcaggctgcagtgctcggcgcagcctgttgtgatgttttcagcctctttggcttccagcaggtaccgttccagcacgcgggagtcgcagatcagtctgggaggagcacactgcacgccttccaggatggccactagaaacacccatcgtagacctagttccatggtggcggatcccggaggctggatcggtcccggtgtcttctatggaggtcaaaacagcgtggatggcgtctccaggcgatctgacggttcactaaacgagctctgcttatatagacctcccaccgtacacgcctaccgcccatttgcgtcaatggggcggagttgttacgacattttggaaagtcccgttgattttggtgccaaaacaaactcccattgacgtcaatggggtggagacttggaaatccccgtgagtcaaaccgctatccacgcccattgatgtactgccaaaaccgcatcaccatggtaatagcgatgactaatacgtagatgtactgccaagtaggaaagtcccataaggtcatgtactgggcataatgccaggcgggccatttaccgtcattgacgtcaatagggggcgtacttggcatatgatacacttgatgtactgccaagtgggcagtttaccgtaaatactccacccattgacgtcaatggaaagtccctattggcgttactatgggaacatacgtcattattgacgtcaatgggcgggggtcgttgggcggtcagccaggcgggccatttaccgtaagttatgtaacgcggaactccatatatgggctatgaactaatgaccccgtaattgattactattaataactagtcaataatcaatgtcatgatcctgacgacggagaccgcggtggttgaccagacaaacctacatcgcgaagcagcgcaaaacgcctaaccctaagcagattcttcatgcaattgtcggtcaagccttgccttgttgtagcttaaattttgctcgcgcactactcagcgacctccaacacacaagcagggagcagatactggcttaactatgcggcatcagagcagattgtactgagagtcgaccataggggatcgggagatctcccgatccgtcgacgtcaggtggcacttttcggggaaatgtgcgcggaacccctatttgtttatttttctaaatacattcaaatatgtatccgctcatgagacaataaccctgataaatgcttcaataatattgaaaaaggaagagtatgagtattcaacatttccgtgtcgcccttattcccttttttgcggcattttgccttcctgtttttgctcacccagaaacgctggtgaaagtaaaagatgctgaagatcagttgggtgcacgagtgggttacatcgaactggatctcaacagcggtaagatccttgagagttttcgccccgaagaacgttttccaatgatgagcacttttaaagttctgctatgtggcgcggtattatcccgtattgacgccgggcaagagcaactcggtcgccgcatacactattctcagaatgacttggttgagtactcaccagtcacagaaaagcatcttacggatggcatgacagtaagagaattatgcagtgctgccataaccatgagtgataacactgcggccaacttacttctgacaacgatcggaggaccgaaggagctaaccgcttttttgcacaacatgggggatcatgtaactcgccttgatcgttgggaaccggagctgaatgaagccataccaaacgacgagcgtgacaccacgatgcctgtagcaatggcaacaacgttgcgcaaactattaactggcgaactacttactctagcttcccggcaacaattaatagactggatggaggcggataaagttgcaggaccacttctgcgctcggcccttccggctggctggtttattgctgataaatctggagccggtgagcgtgggtctcgcggtatcattgcagcactggggccagatggtaagccctcccgtatcgtagttatctacaagagaaactcagtctggtttcactcaggcatgaacccaagcttatgctttgtaaagttcagcttttataggtcaggtcacagtgtgacatctgaggctggtct

SEQ ID NO: 32 - DNA, 22 bp, synthetic construct
  source 1..22: mol_type = other DNA
ctcgacgccatccacgtaccag

SEQ ID NO: 33 - DNA, 8752 bp, synthetic construct
  source 1..8752: mol_type = other DNA
ggtggcccacacctttagtctcagcacttaggaagcagaagcaggtaaatctctgtgagtttgaggacagcctgagctacatagtgagaccctgtttatgaagaaattagaagacaatcctgatgtcaaccggtcttgtgcatgctcacacacaagtgcacacaccctcatacacatacgccatgagcatacacacctgcaaataggaacatccagttctcaggtggtgaaattgagacttgaactggggattgtctggatgccaaagtcaatgctttttatgacaacctaccagtttacaaaggtcgtagtcaagacacaggcctgttggctgctgacaggactgagaaatgaaaggccaactgggtgtccttagtttgaatgggtagagggatgaggtgtgcgcacagctctggagagtgatggctgtgtgacttcagttctgctgggcattggagaaattggaccaattcagagcacttagatttgtgattcaagagttttgattgtccatttggaatagaagaaaccagtgctagtatggagcagttttggtatggggaaaagggacaggaagtcactagtgatgggaagaaagggcagagttcagtttttttctccctggggttttttgtttgtctttttgcttttctttttttttgagacagaatcttgctatgtatagccatagctagcctggaacttactatcttgatcagtctaccttcaaagttggggcaatgctcctgcttccgcccctgccttctgagtgctgggatcaaaggtttgcaccagcatactcagtagctgtaaccaccagcctatcatttattgatgagggtttgtctgctctgggctcagaaccagggactccctttctttatcgaaatgtgtagaactgagttctctccatctccttttttcttctagcagaaactcaggtttttctttctttttctaatttttaacaatgtctcctgaagccgggcggtggtggcgcatgccttcaatcccagcacttgggaggcagaggcaggcggatctctgtgagttcgaggccagcctggtctacaagagctagtttccaggacagcctccaaggccacagataaaccctgtctcgaaaaaaacaaaaaacaacaacaacaacaaaaaagaatgtctcctaaagttctgccgcttccttttcttctgctgctcctgttttctctgcttctgccgcctgagtgctgtgaacgtctctgctaaacatttctgtttagaaccattcacaacactgtcaacctctgagccctcatcccctctggacattcacagcgttaccctccatgctgagggtgctcacctgggcatgcttagtatctcctgggagtctctgggctctttagcagggccctccacagctgtctgagtccacatgagaaaaattaaagccaggtttagatgtcttaaggtctttttcttcatgtccaatggtgtctccagtgccagtatggtcctattacagatactgtcattcgttttgacaagcaggctacctgcgtgtgactcttccctgaagtttctgggttcagctctgtctttctgctctgtagataagcttgccttagtccaagttttaagtcccatttttgtatattgccctcatgtgctcactatccatcatcagtgtggcttctcagaccgtgttcttgcctgtcctgcctaactcttctttttgtttgaacttcttgagagcaagggccattattgctgttgttgttgttggcactaagcacagtataattctagaacacaattcttgaagtccataaatgctaagttttagtctcttttaaaggtacatgatgttgcaatatctcttctttgtggaatgacactctgcatttttttttcagcttcctgttctgatcctgtttgagatggtttaggtttccctttttgtgaaatttgttgctattttaaaataattctgaaggatactcaacaatgatgtctacttattgtctccagatgaaatgagaagttgatcatttattcagtttatcattgggagaaaaggcatctaatactcagcaccacttttattttactgttttttttgtttgtttgttttttgtttttgttttttttttcttgagatggggtttctctgtttaacagccctggctgtcctggaactctctttgtagatcaggctggtctcaaactcatagagatccacctacttctgctttcctaatgctgggactaaagacgtgcaccaccactggctaggataggatctttactatgggtatgtagcccagcctggccttgaccttgtgttagccttcctgcctcagtcatcctgctgagtgccaccataaccaacttctgtcctacctttcagtaccattcctggtctgagtgctttcctacctttttgtcctcagtttcgctctggttctaatctgccaagttttcctgaatgcatggttggcttactgctgatgctctggtcactgccacacagttccagtgctggtgctggggcagcgagacggaagtcttagcagtcggtggtctttgctacacttgacctggctgacaccccactcaaaacttcctttcccacatggcagcgttggggtttgctgctgtttgtgtgtatgtgtgggtatgcggtacaggtatattcacatgtgtaaaagcacctgtgtatacatggaagctgagctgatagtgtcttccttgctcactctgcactttatttactgaggcaggatctctcgctgaacccggaactcaccaattccagctgtcttcccctggcaggcctgtctctgtcgccagagtctggagagaatggtgaccctcatggccaagagcctttgtgtgggttctaatcattaagtattgctgggcgtgtttcattaattcaaaatctaaatggaatgagtgctactttccacaagtctagtctctcaagttgttagtgagcaaggtagctatagggcctgctctcatgcagtttacagtttagatgagaagcatccattcattaatttaattcagtaaatatttacttagtgcctgattttccaagtcctgcttgcctagcaactgaaggtaataatggaaattgtttaattatgtaactgtttaatcttaattgtatcttgaactttaaagaagagatggtgtctctccattggggattagtcccagaaacactactttttcctccagcatacatggatcctcaggttccatatataaagggatccgagtgtttgcatgtaggctcctgtaaaatttaaatatttaaaacatgtatttgtgtgtaggagcatgtggatgtcagagaacaactttgtggagtttgttgtctgtgtgtcccaaggattgatcttgacagcaggcatctttattcactgatgatctagctcctgaccaccttctcctgtatactttaaagtagctggccttacttatgacacgtttaatacagtgtagatgctctagaaattgttgtttaaggaataaaaagtggttctgtacatgttcagcacaggcaactgttcttgttgtttgtttgttttttttttattctgaacattttcactctgtaattgactgaatccatgaatgcagatcccccaggttctgagggctggtggcccaggaagccgtgagagcctagagtaagcctgcctgtcacactcagaactgaggctaaggaccagtctgagagaggcccttgagaaagaaacatcaatagtggagtggctggcctagtacaagaattcagatggagtggggcagggagtgactgcattgcctactgcagccacttacaaagtagtcatctgccatggaaactcaaggatgaaattctgtcctatctcacctctgtgatggaccttacgatggagacagggtcccctttcttacccttcagggatagtgttgaaatttccatttgtaaagttagcacatgtacatgagagactaattaccaatgcaaattaagtgtcgaatgagtggttaacttgcataacactgacatttagaggaggacactgctggatagacatggaggattatggaggaccttggtaggagtgagacttgaattaaagggagaggctctggaaagcaaagaaaggaactagacatttccagtaaagggagaaaagagcacaggaaaggggcgggaactgagagtcaccgaggatgagtgtgctgtgcctctaggcctaggctgaccctcctgctcgcctggttcctgagtcatacagcagaaagtgttgaaaggccctgggaatacccttgatcctacctagacactgggacttttttggtgagaggccttggcgagcaccaagacatatgactgagtgagtcagttgagggaatacagagcacaacctgtgtggcagtgggagggcgatccatgggtaggtgatcaagagcttgtgaaaggtcctattagaagttaaaaagaagaaggggtggggtgggaggaggaaggagtcagtgcccctcccctgtctagcaaactagctgacaggctaaatcccttttaagcctagttgtttgttttgtatagctctagagtactgtttctctacatgtgggtctcgacccctaggggtcaaccagccctttcaaaggggttgccgacgaccattggaaaccacagatacttacattatgattataaaagtggcaaaattacagttatgaagtctcaataaaaacaatcttatggtgggaggtcaccccaacacgaggaactgtattaaaaggatcacacacagcattaggcggttgagaatcactgatctagaactgtttttttttttttttttttttttaacgtgtctgtgaagggcagaggcttcagagtccaggagtgttgggaatgagctctggtcctgcaagagcatcttttcagcccctgtttgtgaggattgaacccagagcctcaggcatgctagacaaacactaactaagccacaactctggcctcagttgttatttgtttaattattttattttggttttttgagacagggttttctgttcaacagacctggctgtcctgtaactcactctgtagaccaggctagcctctgcctccccagttttagaactaaaggcatgaaccatcaccacccagcttattgtattttatttaagtaaagctctcaggtagcctagactggcctagattatctgtatagctaaggatgactgaatgaccttgaatttattgttttatttttgtggcagaatctcactgtatagctctgactggcctggaactctctatgtgagccaaactgacaccaaacttacagaaatggatctgcctctaagcttccaagctctataatcaaggccaccacacctgtccaaccttgaacttttgatactgagtgctgagattcctgacacacccagtttatgtcctgttgggaacagaacccagggcttcatgcatgctgggaaagcactctaccagtgagctgcactccgtcccagttgcaaaaaagatttattgatctttttcagatcaaaataatagttcataatgtgtgaaaattgtatgaaattcaggcttcagtgtccatgaatgtttttggaacatggtagtgttcggttacttgcctgtgacttcttgtaacatgcagggcaagggctgtatagtgacagagaccataaagtccaaaatatcttctctttgacacgacagaaacctgtccaccttgagttatacccacccatccttggctcaaccaccctttctgaaacagaatggtcactgtctcctccctgaggctctgcccttccacccccagccctgattttgtcatctctgtgccaagggccacaccatgttttgttttttattttttgtttctttttttttgtttgtttttttgagacagggtttctctgtgtaacagttttgactgttgtggaactcactctgtagaccaggctggcctctgcctcttttttttttttttttttttttttttttctttttcgagatggggtttctctgtggctttggaggcagtcctggaactagcccttgtagaccaggctggcctcaaactcacagagatcctctgcctctgcctcccaattactgggattaaaggcatgtgtcaccatcacccggctttgttgttttgagacagggtttcactatgtagttctggcaaccttgcatcttactctgtagaccaggctggcctctgcctcttttttttttttttttttttttttttgatttttgggttttcgagacagggtttctctgtggctttggaggctgtcctggaaccagcctggtctcaaacttacagagatcctctgcctctgcctcctgagtgctgggactaaaggcttgtgccaccaccgccctgctggcctctgccttttaagcactagcattaaaggtgtgtaccaccactgccaactgcttcccccctccccctttttttaaccaggtcaatttctctgtgtagtcctagctgtccctgaacttgcttggtagaccaggctggcctcaaactcagatccacctatgtctgcctctcaaatgcagggattaaaagtgtgtgccaccatatatatctcccaccgtatttttttttctccccgagacagggtttctctgtggctttggaggctgacctggaactagctcttgtagaccaggctggtctcgaaatcactgagatccacctgcctctgcctccccagtgctggattaaaggcgtgcgccaccaccgcccggcccttccaccgtattttaagctgcacccaccccactgggctttgtgtgttcttttgaggccttcattcactttcctccaggaattttccctttgttgcggggcagaggtgtgtagtagctcagacattaagacagagtcttgtaattcagccttggctggcctcaaactcagaattcctcttgcttccgcctcccaggcaggcgctaggattacaggtatgcaccaccaccccagctcttggacttttccctctagaaattaagccctcagctcagcccagaagtactggtcctggctctgctctacttctttcatttcaccgctatccggactcccgccccagccttgcagggtctctctgagtcattagggaatccttgtgtgggaatgtatatgtggggggatggggaggtctggttgttttccctgccccgccctttgcttactctgccgtttgtcgttttgatccttttgtttcccatgagacccctcttttagctgctgtgacattccttgctctagctctttctctcacttccttaccaagttctttactagttagtgtgttagatgctgcgtgctccccctgttataattaaacttgtgggggaatttgcgtgggggaccttggcggattccatggcaggcgagggtgacccaggcggagggacaaacatgctaggcagacagcataagtgggaagttttttagaaaggggagggaggaaagagaaaagagctaccttttctaaaagacacagaggacagaagagaagagggagataggaaaatcttgtctgccctaggggaaccctggcaaagaggagctggagagacgggagcagacagagagctggaaaacagaggatccggaaagtgggcggaagtctttgttttaaaggggtcctttgcacctgggctgaccagggtactgcctgagtgcattctgccaggtgacgggcaggccagcttaatgcctgaatccttacacacacacacacacacacacacacgcacacacgcacgcatacacgcatgcacgcgcgcgcgcgcacacacacacatacacacacacactcatcctttgtcctgtggtgtgagctattttataggatactatatgtgtcagttactgtattaaaataccttacataaattattcttaatccattttttgttgttttgtttgtgtttgtttttagtcagggtttcctctagaccaggctggcctcaaacttagagatcagtctgcctctgcctcctgatttctggaattaaaggcatgtgccaccactgctcagcaaatttttcttaatccttgagcagcttttattttattttaacgtttatcccagactgtggtaaggcattcctttcatcccagtattgggaggcagaggtaggcagatctctgtgagttgaaggacagccaaggctattcacagagaaaccctgtcttgaaaagcatatgtatatatacaatttttagttacacataggtttatgactgtatatgggtattttcagggcaagtgcaggtgcccatggagacccagtagctggagtgataggcggttgtgaactgctgggtgtggattcagagaactcaggccctctgtaaagcagtgagtgctcttaactgctgagctgtctctccagctgcctacaacagcttttggaaagatagacttagggcttgggatgtagctcagttggtcaagtgcatgccgtcatacccaaagctggggtcactccctggtactgtatgcaaatctagtgtgctgatacacacgtgtgagctcccagaaggcagaatcaggaggatcggatgtttgaagcctcaagtttgctgtcaacttgtatttcatgagtccctccctgtctcagggtggagaagtgagatctgggcagctgttttcccctactgataaggtatcccatgtcccctgtcag